European Patent Application EP 4 649 964 A1, published November 19, 2025. Title: COMPOSITE LIPID NANOPARTICLE AND preparation method thereof, RNA VACCINE, DRUG AND USE. Applicant: Bisheng (Beijing) Biotechnology Co., Ltd. Application EP. The sequence listing filed with the application follows.

SEQUENCE LISTING (6 sequences)

SEQ ID NO: 1 - DNA, 19 bp, synthetic construct
  source 1..19: mol_type = other DNA
gctgaggccggcatcaccg

SEQ ID NO: 2 - DNA, 46 bp, Synthetic construct
  source 1..46: mol_type = other DNA
aaagatctgctagctcgagtcagtggtggtggtggtggtgatgatg

SEQ ID NO: 3 - DNA, 46 bp, synthetic construct
  source 1..46: mol_type = other DNA
aaagaattcgccaccatggaagttcagctgtctgtgcgtctgaacg

SEQ ID NO: 4 - DNA, 32 bp, Synthetic construct
  source 1..32: mol_type = other DNA
tttgatttccagtttagtaccaccaccgaagg

SEQ ID NO: 5 - DNA, 381 bp, Synthetic construct
  source 1..381: mol_type = other DNA
gctgaggccggcatcaccggcacatggtacaaccagagaggctctacctttaccgtgaccgccggagctgacggtaaccttacaggccagtatgagaaccgcgcacagggctggggctgtcagaatagtccatacacactcacaggtaggtacaacggcaccaagttggaatggagagtggaatggaacaactctaccgagaattgccactccagaaccgagtggagaggccagtaccagggaggtgctgaggccagaatcaatacacagtggaacctgacatacgagggtggcagtggtccagccaccacacagggtcaagacaccttcaccaaggtcaagccttctgctgcatctcatcatcaccaccaccaccaccac

SEQ ID NO: 6 - DNA, 720 bp, Synthetic construct
  source 1..720: mol_type = other DNA
gaagttcagctgtctgtgcgtctgaacggtgaagcgtggggtttctccgaagacagctgcaaagcgtctggttacaccttcaccgactacaacatggactgggttaaacagagccacgaaaagtctctggaatggatcggttacatcaatccgtatagcggtgacaccatctacaaccataaattcaaagataaagcgactctgaccgttgataaatcttccaacatcgcgtacatggaactgcgcagcttgacctctgaagacactgctgtttactactgcgcgcgtggtggttacgattacggtgatcactggggccagggtactactctgactgtgtccagcggttctgcgggtggtggtggttctggtggtggcggtagcggtggcggtggttccgacatcaagatgactcagagtccatcttctatgtacgcaagcctgggtgaacgtgttaccatcacctgcaaagcatctcaagacatcaactcttacctgtcttggttccagcagaaaccgggcaagagtccgaagactctgatctaccgtgccaaccgtctggtaggcggtgtaccgtctcgtttctccggttctggttccggtcaagactacagcctgaccatcagcagcctggaatatgaagacatgggcatctactactgcctgcaagacgacgaatttccgcgtaccttcggtggtggtactaaactggaaatcaaa